European Patent Specification EP 3 881 850 B1, published July 17, 2024. Title: A composition for inhibiting replication of hepatitis B virus. Applicant: Tokyo Metropolitan Institute of Medical Science. The sequence listing filed with the application follows.

SEQUENCE LISTING (22 sequences)

SEQ ID NO: 1 - RNA, 20 nt, Artificial
  Synthetic RNA
gagcuuggucuguagcgguu

SEQ ID NO: 2 - DNA, 20 bp, Artificial
  Synthetic DNA
aaccgctacagaccaagctc

SEQ ID NO: 3 - RNA, 20 nt, Artificial
  Synthetic RNA
cacugccuuccaccaaacuc

SEQ ID NO: 4 - RNA, 20 nt, Artificial
  Synthetic RNA
gagcuuggucuguagcgguu

SEQ ID NO: 5 - DNA, 19 bp, Artificial
  Synthetic RNA
uaccgcuguuaccaauuuu

SEQ ID NO: 6 - RNA, 20 nt, Artificial
  Synthetic RNA
gagcuuggucuguagcgguu

SEQ ID NO: 7 - RNA, 22 nt, Artificial
  Synthetic RNA
cacuguucaagccuccaagcug

SEQ ID NO: 8 - RNA, 20 nt, Artificial
  Synthetic RNA
gagcuuggucuguagcgguu

SEQ ID NO: 9 - RNA, 23 nt, Artificial
  Synthetic RNA
uggaugaugugguauugggggcc

SEQ ID NO: 10 - RNA, 22 nt, Artificial
  Synthetic RNA
agccccugcccaccgcacacug

SEQ ID NO: 11 - RNA, 21 nt, Artificial
  Synthetic RNA
acuccaccauagaucacuccc

SEQ ID NO: 12 - RNA, 22 nt, Artificial
  Synthetic RNA
uggagugugacaaugguguuug

SEQ ID NO: 13 - DNA, 61 bp, Artificial
  Synthetic DNA
tgtacatgtcccactgttcaagcctccaagctgtgccttgggtggctttggggcatggaca

SEQ ID NO: 14 - DNA, 61 bp, Artificial
  Synthetic DNA
tgtacatgtcccacttttcaagcctccaagctgtgccttgggtggctttggggcatggaca

SEQ ID NO: 15 - DNA, 61 bp, Artificial
  Synthetic DNA
tgttcatgtcctactgttcaagcctccaagctgtgccttgggtggctttggggcatggaca

SEQ ID NO: 16 - DNA, 61 bp, Artificial
  Synthetic DNA
tgttcatgtcctactgttcaagcctccaagctgtgccttgggtggctttagggcatggaca

SEQ ID NO: 17 - DNA, 61 bp, Artificial; identical to SEQ ID NO: 15
  Synthetic DNA

SEQ ID NO: 18 - DNA, 61 bp, Artificial; identical to SEQ ID NO: 15
  Synthetic DNA

SEQ ID NO: 19 - DNA, 61 bp, Artificial; identical to SEQ ID NO: 15
  Synthetic DNA

SEQ ID NO: 20 - DNA, 61 bp, Artificial; identical to SEQ ID NO: 15
  Synthetic DNA

SEQ ID NO: 21 - DNA, 61 bp, Artificial; identical to SEQ ID NO: 15
  Synthetic DNA

SEQ ID NO: 22 - DNA, 61 bp, Artificial; identical to SEQ ID NO: 15
  Synthetic DNA